European Patent Application EP 4 516 900 A1, published March 5, 2025. Title: EROLIDOL SYNTHASE AND USE THEREOF. Applicant: WUHAN HESHENG TECHNOLOGY CO., LTD. Application EP. The sequence listing filed with the application follows.

SEQUENCE LISTING (119 sequences)

SEQ ID NO: 1 - protein, 531 aa, synthetic construct
MIINNCVTPKDTQPAPLPSETDIVSNDINIKNELSLKHLELLEEVRYLLKNYSSEPLDMVDALQKLCINHYYEDEIGLILKLLYARMSNNGDYKHDKSLYEVSLSFRILRQEGYYVSADVFADFKQKDGKFKEEIAQDVKGLMALYEASQLSLDGERILEEASDFSSGALKDMVPSLDLHQAMIATNTLQHTYQRTSSTFMVKKFMKVYTGTPMCELAQLELTTKVQSLHRTELEQISRWWKDLGLAQELKLARNQPLHWYLWPMASLTDLSLSEQRIELTKPIAFIFLIDDIFDVYGTLDQLVILTQAVNRWESNSLERLPHHLRICIQALFDVTNEISDNIYKKHGFNPIDFLKQSWINLCEAFLVEAKWFAEGYMPTAEDYLNNGMVSTGAHVVIVHMFFLLGGGPNIKSASVVNENQGITSCLAKILRLWDDLGSAEDVDQDGNDGSYVTYYMKENAGCSIQKAHEHVMEMISNTWKQLNAECLYSSHLSRTFTKACLNLARMIPMMYDYDENHSLPFIKEYINSMF

SEQ ID NO: 2 - protein, 571 aa, synthetic construct
MAPPPSSYPPSARNNFTQVGTGLSDTMNEPSTQKWSITSHDGTLVSSPIILHNSKANNACYTDEFHVDHESKLNEVRDLLNKVGEDYQLEGLVMIDAIQCLNIDYRFRKEIESILQSQDETSRVHENDEHDLYQTALRFRLLRQEGHFVSAEVFDKFKNKEGKFKQELVEDIRGMMGLYEAAQLRIEGEHILDEAESFCRRLFKGCMPYLNSHEAKLVESTLKHPYRKSLSRIGAKNFANNFQGNFKWITVLEELSNLDLKIVQSIHQKELQQISHWWEELGLAKELKLARDQPLKWHMWSMEVLQDPSLSEQRIELTKPISLVYIIDDIFDVYGTLDELTLFTEAVTRWEFTDANQLPNYMRTCFQTLFDITYEIGYKFFIVHGWNPIDTLRKSWVTLCKAFLAEAKWFASGELPKADKYLKNGIISSGVHVVLVHMFFLLGQDLTKECLDLVNDNNNIPGIINYTATILRLWDDLGSAKDENQDGYDGSYLECFMNEHKGLLMKTAREHMIGMISDAWKCLNKECLSPNPFSSSFTKASLNAARMVPLMYNYDDNHCLPDLEEHIQCLF

SEQ ID NO: 3 - protein, 528 aa, synthetic construct
MTISVTRKDTQPTPFPSETDIVSNDINIKNELSIRHLELLEEVRNLLKNCSSKPLVMVDTLQKLCINHHYEEEIGLILKSLYTRMSNNDDYKHDKSLYEVSLSFRILRQHGYYVSADVFANFKQKDGKFKGEITQDLKGLIALYEASQLSLEGEQILKEASDFSSGALKEMMPSLDQDQAMIVTNTLQHTYQRTTSTFMVKKFMKVYTGTPMCELAQLELTKVQSLHRTEVDQISRWWKGLGLAQELKLARNQPLHWYLWPMASLTDLSLSEQRVELTKPIAFIFLIDDIFDVYGTLDQLVILTQAVNRWESNRLEQLPYHLRICIQALFDVTNEISDKIYKKHGFNPIEFLKQSWINLCDAFLVEAKWFAEGYMPTAEDYLNNGMVSTGVHVVIVHMFFLLGGGPNIKSASVVNENQGIMSCLAKILRLWDDLGSAKDVDQDGNDGSYVTYYMKENAGCSIQKAHEHVMEMISNTWKQLNAECLYSSHFSRTFTKACLNLAKMIPMMYDYDENHSLPFIEEYINSMF

SEQ ID NO: 4 - protein, 525 aa, synthetic construct
MSINILHGDLPDVKVMSPQADATEKIDELKEKIRRVLMTTSDPKMSLKLVDTIQRLRIGYYFQEDINEILEKLKQCLPDDELHIVALCFRLLRQNGIPTNSEVFRKFIDMNGEFIKSTSEDIEGLLSLYEASYMGSNEEIFLVHAKKITTRELNICVPKLSPKLSKKVLQALELPMHLRMETLEARRYIEDYGNEEDHNPLLLELAKLDYNHVQSLFRRELVEMARWWNHLGIARKFSFVRDRHVECFLWTVGVLPEPKYSATRIVMAKITSILLLLDDIYDTYGSYDDLVLLTKIIQRWDMTEIEQLPEYMQACYMALYNTTSEICDKVLRERGLYVEQFLRKTWIKIVEGYMVEVKWLKTGTIPNFKEYMDNAVTTSGSYMAFVHMFFLICDEVNKENMADLLEPYPKFFTLAGTILRLWDDLGTVKEEQERGEVLSSIQLLMKEKKITCDKDERKQILELIHELWKDLNAELVAPNAVLWPMIRVALNMSRTSQVVYQHNEDSYLSSVKDHVKNLFFKAIDM

SEQ ID NO: 5 - DNA, 1596 bp, synthetic construct
  source 1..1596: mol_type = other DNA
atgatcatcaacaattgtgttacaccgaaagacacccagccagcccctctcccatctgaaacagatattgtgtcaaatgacattaacattaagaatgaattgtccctcaaacatctagaattgttagaagaagtccgatatcttctaaagaattattcttccgaacctttggacatggttgacgctcttcaaaaactttgcatcaaccattactatgaagacgagattggcttgattttgaaattgctctacgctagaatgtcgaataatggcgactacaagcatgataaaagtctttatgaggtttccctttcttttcgcatccttcgtcaagaaggttactatgtctcagctgatgtttttgctgatttcaaacaaaaggatgggaagtttaaagaagaaatagcacaagatgttaagggtctaatggcgttatatgaagcttcacagctaagcctggatggagaacgaatacttgaagaggcttcagattttagcagtggtgctcttaaagacatggtgccttctttagatctacatcaagctatgattgctactaacacattacaacatacgtatcaaagaacctcatcaactttcatggttaaaaaattcatgaaagtatacacgggtacacccatgtgtgaactagcccaattagagttgactactaaagtccagtcactacatcgaacagaactagaacaaatctccagatggtggaaggacttggggttggcgcaagagttgaagcttgcaagaaaccaaccgttgcactggtacttatggccaatggctagcctcacagatctcagcttgtccgagcagagaattgagctcacgaagcccattgctttcatctttctaattgatgacatttttgatgtttatggaactctagaccaacttgttatcttgacacaagcagtgaatagatgggaaagtaacagccttgaacgactcccacatcacctaaggatctgtattcaagctctatttgacgtaacaaacgaaataagtgacaatatctacaagaagcatgggttcaatcccattgattttttgaaacaatcgtggataaacctttgtgaagcttttctagtagaggcgaaatggtttgctgagggatacatgccgacggcagaggattacttgaataatgggatggttagtacaggggcacatgtcgtgatagtgcacatgttcttcctcctcggtggtggccctaacataaaaagtgctagcgttgtaaacgaaaaccaagggattacgtcttgtttggcaaagattcttcgtctttgggatgacttaggaagtgctgaggatgtggatcaagacggtaatgatggatcatatgtgacatattacatgaaagagaatgcaggttgttctattcaaaaggcacatgaacatgttatggaaatgatatcgaatacttggaagcaactaaatgcggagtgcctttactcaagtcatttatcacgtacattcaccaaagcttgcctcaatcttgcaagaatgattccaatgatgtacgattatgatgagaatcattcccttcctttcatcaaggaatatataaactccatgttttaa

SEQ ID NO: 6 - DNA, 1716 bp, synthetic construct
  source 1..1716: mol_type = other DNA
atggcaccccctccttcctcctatcctccaagtgctcgaaacaattttacacaagttggcacaggacttagtgatacgatgaacgagccttctactcagaaatggagcattaccagccatgatggcaccttagtttcaagccctataatacttcacaactctaaagcaaacaatgcttgttatactgatgaatttcatgtcgatcatgaaagcaaattgaatgaagttagggatttgcttaacaaagttggagaagattatcaattagaaggtttggtcatgatcgacgccattcaatgcctaaacattgactatcgcttccgaaaggagattgagtccatcctacaaagtcaggatgagacatctagggttcatgaaaatgatgaacacgatctttaccagactgcacttcgttttcgactgctgagacaagaaggccattttgtgtctgcagaagtgtttgacaaattcaagaacaaagaggggaagtttaagcaagaactagttgaagatataaggggaatgatgggcttatatgaagctgcgcagcttagaattgaaggagaacatatacttgatgaagccgaaagcttttgtcgtcggctctttaaaggatgcatgccctatcttaactctcatgaagcaaaacttgtcgagagcacgctaaagcatccctatcgaaagagcttgtcacgcataggggccaaaaacttcgctaacaatttccaaggcaattttaaatggattactgttcttgaagaactatcaaatttagatttgaaaatagttcaatctatacaccagaaggaactacaacaaatttcccattggtgggaagaacttggtttagcaaaggaattgaagctcgcaagagaccaaccgctaaaatggcacatgtggtccatggaagtgttacaagatccaagcttgtctgagcaaaggattgagcttacaaagcccatttctcttgtatacataattgatgacattttcgacgtttatgggacgcttgatgaactcactctcttcacggaagcagtcactagatgggaattcaccgacgcaaatcaactgcctaactacatgaggacatgtttccagactctctttgatatcacttatgaaattggctacaagtttttcatagttcatggttggaaccctatagacacactacgaaaatcgtgggttactttgtgcaaagcatttttggcggaagcaaaatggtttgcttctggggaattgccaaaggcagataaatacttgaaaaatggaattattagttcaggagtgcatgtagtacttgttcacatgttttttctcttgggtcaagatttaacaaaggaatgtttagacctagtgaacgacaacaacaatattccaggcatcataaactatacggcaacgattcttcgtctttgggatgacttgggaagtgcaaaggatgagaatcaagatgggtacgacggatcatatctggaatgtttcatgaatgaacacaaaggtttattaatgaagactgcaagagagcatatgattggcatgatttcggatgcatggaagtgcttgaacaaggaatgcctctctccaaatccattttcatcatctttcacaaaggcttctcttaatgctgcaaggatggttccattgatgtacaattacgacgacaaccattgtctcccagatcttgaggagcatatacaatgtttgttttaa

SEQ ID NO: 7 - DNA, 1587 bp, synthetic construct
  source 1..1587: mol_type = other DNA
atgacaatctctgttactagaaaggatactcaaccaacaccatttccatctgaaactgatattgtttctaacgatatcaacatcaagaacgaattgtctattagacatttggaattgttggaagaagttagaaatttgttgaagaactgttcttctaagccattagttatggttgatactttacaaaagctgtgtattaaccatcattacgaagaagaaatcggtttgattttgaaatctttgtacacaagaatgtccaataacgatgattataagcatgataagtccttatacgaagtttctttgtcttttagaatcttgagacaacatggttattacgtttctgctgatgtttttgctaattttaagcaaaaggacggtaaatttaagggtgaaattacacaagatctgaaaggtttaatcgctttatatgaagctagtcaattgtctttggaaggtgaacaaattttaaaggaagctagtgatttctcttctggtgctttgaaagaaatgatgccatctttggatcaagatcaagctatgattgttacaaatactttgcaacatacctaccaaagaacaacttctacttttatggttaagaagttcatgaaggtttacactggtacaccaatgtgtgaattggctcaattggaattgactaaagttcaatctttgcatagaacagaagttgatcaaatttctagatggtggaaaggtttaggtttggctcaagaattaaaattagctagaaaccaaccattgcattggtatttatggccaatggcttctttgactgatttgtctttgtctgaacaaagagttgaattgactaagccaattgcttttattttcttgatcgatgatatcttcgacgtttatggtactttggatcaattagttatcttgactcaagctgttaatagatgggaatctaatagattagagcaattaccataccatttgagaatttgtatccaagctctatttgatgttacaaatgaaatctctgacaagatttacaagaagcatggttttaatccaatcgaatttttgaagcaatcctggattaatttgtgtgatgcttttttggttgaggctaaatggtttgctgaaggttatatgccaactgctgaagattatttaaacaatggtatggtttccacaggtgttcatgttgttattgttcatatgtttttcctgttgggtggtggtccaaatattaaatctgcttctgttgttaacgagaatcaaggtattatgtcttgtttggctaaaattttgaggttatgggatgatttaggttctgctaaagatgttgatcaagatggtaatgatggttcttatgttacatattacatgaaggaaaacgctggttgttctattcaaaaagctcatgaacatgttatggaaatgatttctaacacttggaaacaattgaacgctgaatgtttatattcctctcatttttctaggacattcactaaagcatgtttgaatttggctaaaatgatcccaatgatgtatgattatgacgaaaatcattccttgccatttattgaagaatacattaactccatgttctaa

SEQ ID NO: 8 - DNA, 1578 bp, synthetic construct
  source 1..1578: mol_type = other DNA
atgtctatcaacatcttgcatggtgatttgccagatgttaaagttatgtctccacaagctgatgctacagaaaaaattgatgaattaaaggagaagatcaggagagttttgatgactacatctgatccaaaaatgtctttaaagttggttgatactatccaaagattgagaattggttattacttccaagaagatatcaacgaaatcttggaaaaattgaagcaatgtttgccagatgatgaattgcatattgttgctttgtgttttagattgttgagacaaaatggtatcccaacaaattctgaagtttttagaaagttcatcgacatgaatggtgaatttattaagtctacttccgaagatatcgaaggtttgttatctttgtatgaagctagttatatgggttctaatgaagaaattttcctggttcatgctaaaaaaatcacaactagagaattgaacatctgtgttccaaaattgtctccaaaattgtcaaaaaaggtcttgcaagctctagaattgccaatgcatttgagaatggaaacattggaagctagaagatatattgaagattacggtaatgaggaagatcataatccattattactggaattggctaaattggattacaatcatgttcaatctctgtttagaagagaattagttgaaatggctagatggtggaatcatttgggtattgctagaaaattttcctttgttagagacagacatgttgaatgttttttgtggactgttggtgttttgccagaaccaaaatattctgctactagaattgttatggctaaaattacttccatcttgttattgttggacgatatttatgacacttacggttcttatgatgatttggttttattgacaaagatcatccaaagatgggatatgacagaaattgaacaattgccagaatatatgcaagcatgttatatggctttgtataatactacatccgaaatttgtgacaaggttttaagagaaagaggtttgtatgttgaacaatttttgagaaagacctggattaaaatcgttgaaggttatatggttgaggttaaatggttaaaaaccggtactattccaaattttaaggaatatatggacaacgctgttactacttctggttcttatatggcttttgttcatatgtttttcctgatttgtgacgaagttaataaggaaaatatggctgatttgttggaaccatatccaaaatttttcactttggctggtacaattttgagattgtgggatgatttaggtactgttaaagaagaacaagaaagaggtgaagttttgtcttctattcaattattgatgaaggagaagaagatcacttgtgataaagatgaaagaaagcaaatcttggaattgattcatgaattgtggaaagatttgaacgctgaattagttgctccaaatgctgttttgtggccaatgattagagttgctttaaatatgtctaggacatctcaagttgtttatcaacataatgaggattcttacttgtcttctgttaaagatcatgttaagaacttgttcttcaaggctattgatatgtaa

SEQ ID NO: 9 - DNA, 1734 bp, synthetic construct
  source 1..1734: mol_type = other DNA
atggcaccccctccttcctcctatcctccaagtgctcgaaacaattttacacaagttggcacaggacttggtgatacgatgaacgagccttctactcagaaatggagcattaccagccatgatggcaccttagtttcaagccctataatacttcacaactctaaagcaaacaatgcttgttatactgatgaatttcatgtcgatcatgaaagaaaattgaatgaagttagggatttgcttaacaaagttggagaagattatcaattagaaggtttggtcatgatcgacgccattcaatgcctaaacattgactatcacttccgaaaggagattgagtccatcctacaatgtcaggatgagacatctagggttcatgaaaatgatgaacacgatctttaccagactgcacttcgttttcgactgctgagacaagaaggccattttgtgtctgcagaagtgtttgacaaattcaagaacaaagaggggaagtttaagcaagaactagttgaagatataaggggaatgatgggcttatatgaagctgcgcagcttagaattgaaggagaacatatacttgatgaagccgaaagcttttgtcgtcggctctttaaagcatgcatgccctatcttaactctcatgaagcaagacttgtcgagagcatgataaagcatccctatcgaaagagcttgtcacgcataggggccaaaaacttcgctaacaatttccaaggcaatttcaaatggattactgttcttgaagaactatcaaatttagatttgaaaatagttcaatctatacaccagaaggaactacaacaaatttcccattggtgggaagaactgggtttagcaaaggaattgaagctcgcaagagaccaaccgctaaaatggcacatgtggtccatggaagtgttaacagatccaagcttgtctgagcaaaggattgagcttacaaagcccatttctcttgtatacataattgatgacattttcgacgtttatgggacgcttgatgaactcactctcttcacggaagcagtcacaagatgggaattcaccgacgtaaatcaactgcctaactacatgaggacatgtttccagactctctttgatatcacttatgaaattggctataagtttttcatagttcatggttggaaccctataaacacactacgaaaatcgtgggttactttgtgcaaagcatttttggcggaagcaaaatggtttgcttctggggaattgccaaaggcagataaatacttgaaaaatgggattattagttcaggagtgcatgtagtacttgttcacatgttttttctcttgggtcaagatttaacaaaggaatgtttagacctagtgaacgacaacaacaatattccaggcatcataaactatacggcaacgattcttcgtctttgggatgacttgggaagtgcaaaggatgagaatcaagacgggtacgacggatcatatctggaatgtttcatgaatgaacacaaaggtttattaatgaagactgcaagagagcatatgattggcatgatttcggatgcatggaagtgcttgaacaaggaatgcctctctccaaatccattttcatcatctttcacaaaggcttctcttaatgctgcaaggatggttcctttgatgtacaattacgacgacaaccattgtctcccagatcttgaggaacatgcaatgtttgttttaaatatgataaacgttacatag

SEQ ID NO: 10 - DNA, 1734 bp, synthetic construct
  source 1..1734: mol_type = other DNA
atggcaccccctccttcctcctatcctccaagtgctcgaaacaattttacacaagttggcacaggacttggtgatacgatgaacgagccttctactcagaaatggagcattaccagccatgatggcaccttagtttcaagccctataatacttcacaactctaaagcaaacaatgcttgttatactgatgaatttcatgtcgatcatgaaagaaaattgaatgaagttagggatttgcttaacaaagttggagaagattatcaattagaaggtttggtcatgatcgacgccattcaatgcctaaacattgactatcacttccgaaaggagattgagtccatcctacaatgtcaggatgagacatctagggttcatgaaaatgatgaacacgatctttaccagactgcacttcgttttcgactgctgagacaagaaggccattttgtgtctgcagaagtgtttgacaaattcaagaacaaagaggggaagttcaagcaagaactagttgaagatataaggggaatgatgggcttatatgaagctgcgcagcttagaattgaaggagaacatatacttgatgaagccgaaagcttttgtcgtcggctctttaaagcatgcatgccctatcttaactctcatgaagcaagacttgtcgagagcatgataaagcatccctatcgaaagagcttgtcccgcataggggccaaaaacttcactaacaatttccaaggcaatttcaaatggattactgttcttgaagaactatcaaatttagatttgaaaatagttcaatctatacaccagaaggaactacaacaaatttcccattggtgggaagaactgggtttagcaaaggaattgaagctcgcaagagaccaaccgctaaaatggcacatgtggtccatggaagtgttaacagatccaagcttgtctgagcaaaggattgagcttacaaagcccatttctcttgtatacataattgatgacattttcgacgtttatgggacgcttgatgaactcactctcttcacggaagcagtcacaagatgggaattcaccgacgtaaatcaactgcctaactacatgaggacatgtttccagactctctttgatatcacttatgaaattggctacaagtttttcatagttcatggttggaaccctatagacacactacgaaaatcgtgggttactttgtgcaaagcatttttggcggaagcaaaatggtttgcttctggggaattgccaaaggcagataaatacttgaaaaatgggattattagttcaggagtgcatgtagtacttgttcacatgttttttctcttgggtcaagatttatcaaaggaatgtttagacctagtgaacgacaacaacaatattccaggcatcataaactatacggcaacgattcttcgtctttgggatgacttgggaagtgcaaaggatgagaatcaagacgggtacgacggatcatatctggaatgtttcatgaatgaacacaaaggtttattaatgaagactgcaagagagcatatgattggcatgatttcggatgcatggaagtgcttgaacaaggaatgcctctctccaaatccattttcatcatctttcacaaaggcttctcttaatgctgcaaggatggttcctttgatgtacaattacgacgacaaccattgtctcccagatcttgaggaacatgcaatgtttgttttaaatatgataaacgttacatag

SEQ ID NO: 11 - protein, 577 aa, synthetic construct
MAPPPSSYPPSARNNFTQVGTGLGDTMNEPSTQKWSITSHDGTLVSSPIILHNSKANNACYTDEFHVDHERKLNEVRDLLNKVGEDYQLEGLVMIDAIQCLNIDYHFRKEIESILQCQDETSRVHENDEHDLYQTALRFRLLRQEGHFVSAEVFDKFKNKEGKFKQELVEDIRGMMGLYEAAQLRIEGEHILDEAESFCRRLFKACMPYLNSHEARLVESMIKHPYRKSLSRIGAKNFANNFQGNFKWITVLEELSNLDLKIVQSIHQKELQQISHWWEELGLAKELKLARDQPLKWHMWSMEVLTDPSLSEQRIELTKPISLVYIIDDIFDVYGTLDELTLFTEAVTRWEFTDVNQLPNYMRTCFQTLFDITYEIGYKFFIVHGWNPINTLRKSWVTLCKAFLAEAKWFASGELPKADKYLKNGIISSGVHVVLVHMFFLLGQDLTKECLDLVNDNNNIPGIINYTATILRLWDDLGSAKDENQDGYDGSYLECFMNEHKGLLMKTAREHMIGMISDAWKCLNKECLSPNPFSSSFTKASLNAARMVPLMYNYDDNHCLPDLEEHAMFVLNMINVT

SEQ ID NO: 12 - protein, 577 aa, synthetic construct
MAPPPSSYPPSARNNFTQVGTGLGDTMNEPSTQKWSITSHDGTLVSSPIILHNSKANNACYTDEFHVDHERKLNEVRDLLNKVGEDYQLEGLVMIDAIQCLNIDYHFRKEIESILQCQDETSRVHENDEHDLYQTALRFRLLRQEGHFVSAEVFDKFKNKEGKFKQELVEDIRGMMGLYEAAQLRIEGEHILDEAESFCRRLFKACMPYLNSHEARLVESMIKHPYRKSLSRIGAKNFTNNFQGNFKWITVLEELSNLDLKIVQSIHQKELQQISHWWEELGLAKELKLARDQPLKWHMWSMEVLTDPSLSEQRIELTKPISLVYIIDDIFDVYGTLDELTLFTEAVTRWEFTDVNQLPNYMRTCFQTLFDITYEIGYKFFIVHGWNPIDTLRKSWVTLCKAFLAEAKWFASGELPKADKYLKNGIISSGVHVVLVHMFFLLGQDLSKECLDLVNDNNNIPGIINYTATILRLWDDLGSAKDENQDGYDGSYLECFMNEHKGLLMKTAREHMIGMISDAWKCLNKECLSPNPFSSSFTKASLNAARMVPLMYNYDDNHCLPDLEEHAMFVLNMINVT

SEQ ID NO: 13 - DNA, 59 bp, synthetic construct
  source 1..59: mol_type = other DNA
actaaagggaacaaaagctggagctctagtagtttaaacataacgagaacacacagggg

SEQ ID NO: 14 - DNA, 53 bp, synthetic construct
  source 1..53: mol_type = other DNA
cattaaagtaacttaaggagttaaatttaagcaaggattttcttaacttcttc

SEQ ID NO: 15 - DNA, 56 bp, synthetic construct
  source 1..56: mol_type = other DNA
gaagttaagaaaatccttgcttaaatttaactccttaagttactttaatgatttag

SEQ ID NO: 16 - DNA, 41 bp, synthetic construct
  source 1..41: mol_type = other DNA
tcgaaggctttaatttgcgcgaaaagccaattagtgtgata

SEQ ID NO: 17 - DNA, 46 bp, synthetic construct
  source 1..46: mol_type = other DNA
tagtatcacactaattggcttttcgcgcaaattaaagccttcgagc

SEQ ID NO: 18 - DNA, 49 bp, synthetic construct
  source 1..49: mol_type = other DNA
gggacgcgccctgtagcggctgaggtctcaacaggccccttttcctttg

SEQ ID NO: 19 - DNA, 55 bp, synthetic construct
  source 1..55: mol_type = other DNA
catgatatcgacaaaggaaaaggggcctgttgagacctcagccgctacagggcgc

SEQ ID NO: 20 - DNA, 52 bp, synthetic construct
  source 1..52: mol_type = other DNA
gaatttttgaaaattcaatataaatgtgagaccaccatgattacgccaagcg

SEQ ID NO: 21 - DNA, 57 bp, synthetic construct
  source 1..57: mol_type = other DNA
taatcatggtggtctcacatttatattgaattttcaaaaattcttactttttttttg

SEQ ID NO: 22 - DNA, 62 bp, synthetic construct
  source 1..62: mol_type = other DNA
atctctctctcctaatttctttttctgaagccattatagttttttctccttgacgttaaagt

SEQ ID NO: 23 - DNA, 50 bp, synthetic construct
  source 1..50: mol_type = other DNA
ttaacgtcaaggagaaaaaactataatggcttcagaaaaagaaattagga

SEQ ID NO: 24 - DNA, 59 bp, synthetic construct
  source 1..59: mol_type = other DNA
atgtacaaatatcataaaaaaagagaatctttttaaaaaaaatccttggactagtcacg

SEQ ID NO: 25 - DNA, 59 bp, synthetic construct
  source 1..59: mol_type = other DNA
actagtccaaggattttttttaaaaagattctctttttttatgatatttgtacataaac

SEQ ID NO: 26 - DNA, 59 bp, synthetic construct
  source 1..59: mol_type = other DNA
gcgccattcgccattcaggctgcgcaactgttgtttaaacgacaacgaccaagctcaca

SEQ ID NO: 27 - DNA, 50 bp, synthetic construct
  source 1..50: mol_type = other DNA
gatgtgagcttggtcgttgtcgtttaaacaacagttgcgcagcctgaatg

SEQ ID NO: 28 - DNA, 59 bp, synthetic construct
  source 1..59: mol_type = other DNA
tcaacagtatagaaccgtggatgatgtggtttctacaggatctgacattattattgttg

SEQ ID NO: 29 - DNA, 59 bp, synthetic construct
  source 1..59: mol_type = other DNA
atagtcctcttccaacaataataatgtcagatcctgtagaaaccacatcatccacggtt

SEQ ID NO: 30 - DNA, 59 bp, synthetic construct
  source 1..59: mol_type = other DNA
agggcttaccatctggccccagtgctgcaatgataccgcgcgacccacgctcaccggct

SEQ ID NO: 31 - DNA, 59 bp, synthetic construct
  source 1..59: mol_type = other DNA
tgataaatctggagccggtgagcgtgggtcgcgcggtatcattgcagcactggggccag

SEQ ID NO: 32 - DNA, 59 bp, synthetic construct
  source 1..59: mol_type = other DNA
cgatagcgcccctgtgtgttctcgttatgtttaaactactagagctccagcttttgttc

SEQ ID NO: 33 - DNA, 51 bp, synthetic construct
  source 1..51: mol_type = other DNA
acaaaggaaaaggggcctgtttaaaacatggagtttatatattccttgatg

SEQ ID NO: 34 - DNA, 45 bp, synthetic construct
  source 1..45: mol_type = other DNA
tttttgaaaattcaatataaatgatcatcaacaattgtgttacac

SEQ ID NO: 35 - DNA, 50 bp, synthetic construct
  source 1..50: mol_type = other DNA
acaaaggaaaaggggcctgtttaaaacaaacattgtatatgctcctcaag

SEQ ID NO: 36 - DNA, 38 bp, synthetic construct
  source 1..38: mol_type = other DNA
tttttgaaaattcaatataaatggcaccccctccttcc

SEQ ID NO: 37 - DNA, 55 bp, synthetic construct
  source 1..55: mol_type = other DNA
acaaaggaaaaggggcctgtctatgtaacgtttatcatatttaaaacaaacattg

SEQ ID NO: 38 - DNA, 38 bp, synthetic construct; identical to SEQ ID NO: 36
  source 1..38: mol_type = other DNA

SEQ ID NO: 39 - DNA, 55 bp, synthetic construct; identical to SEQ ID NO: 37
  source 1..55: mol_type = other DNA

SEQ ID NO: 40 - DNA, 38 bp, synthetic construct; identical to SEQ ID NO: 36
  source 1..38: mol_type = other DNA

SEQ ID NO: 41 - DNA, 66 bp, synthetic construct
  source 1..66: mol_type = other DNA
ggaaaaggggcctgtttacttatcgtcgtcatccttgtaatcgaacatggagttaatgtattcttc

SEQ ID NO: 42 - DNA, 43 bp, synthetic construct
  source 1..43: mol_type = other DNA
gaatttttgaaaattcaatataaatgacaatctctgttactag

SEQ ID NO: 43 - DNA, 67 bp, synthetic construct
  source 1..67: mol_type = other DNA
ggaaaaggggcctgtttacttatcgtcgtcatccttgtaatccatatcaatagccttgaagaacaag

SEQ ID NO: 44 - DNA, 45 bp, synthetic construct
  source 1..45: mol_type = other DNA
gaatttttgaaaattcaatataaatgtctatcaacatcttgcatg

SEQ ID NO: 45 - DNA, 59 bp, synthetic construct
  source 1..59: mol_type = other DNA
attaaccctcactaaagggaacaaaagcgtttaaacacgcagataattccaggtatttt

SEQ ID NO: 46 - DNA, 54 bp, synthetic construct
  source 1..54: mol_type = other DNA
aatacgactcactatagggcgaattgggtaccttcgtttcctgcaggtttttgt

SEQ ID NO: 47 - DNA, 46 bp, synthetic construct
  source 1..46: mol_type = other DNA
caaaaacctgcaggaaacgaaggtacccaattcgccctatagtgag

SEQ ID NO: 48 - DNA, 50 bp, synthetic construct
  source 1..50: mol_type = other DNA
gttttgggacgctcgaaggctttaatttgctcacagcttgtctgtaagcg

SEQ ID NO: 49 - DNA, 59 bp, synthetic construct
  source 1..59: mol_type = other DNA
ttgtctgctcccggcatccgcttacagacaagctgtgagcaaattaaagccttcgagcg

SEQ ID NO: 50 - DNA, 59 bp, synthetic construct
  source 1..59: mol_type = other DNA
gtttgaaagatgggtccgtcacctgcattaaatcctaaacaggccccttttcctttgtc

SEQ ID NO: 51 - DNA, 59 bp, synthetic construct
  source 1..59: mol_type = other DNA
taattacatgatatcgacaaaggaaaaggggcctgtttaggatttaatgcaggtgacgg

SEQ ID NO: 52 - DNA, 49 bp, synthetic construct
  source 1..49: mol_type = other DNA
gaatttttgaaaattcaatataaatggttttaaccaataaaacagtcat

SEQ ID NO: 53 - DNA, 58 bp, synthetic construct
  source 1..58: mol_type = other DNA
gttttattggttaaaaccatttatattgaattttcaaaaattcttactttttttttgg

SEQ ID NO: 54 - DNA, 50 bp, synthetic construct
  source 1..50: mol_type = other DNA
taacacaattgttgatgatcattatagttttttctccttgacgttaaagt

SEQ ID NO: 55 - DNA, 45 bp, synthetic construct
  source 1..45: mol_type = other DNA
gtcaaggagaaaaaactataatgatcatcaacaattgtgttacac

SEQ ID NO: 56 - DNA, 51 bp, synthetic construct
  source 1..51: mol_type = other DNA
cgatttcaattcaattcaatttaaaacatggagtttatatattccttgatg

SEQ ID NO: 57 - DNA, 51 bp, synthetic construct
  source 1..51: mol_type = other DNA
tatataaactccatgttttaaattgaattgaattgaaatcgatagatcaat

SEQ ID NO: 58 - DNA, 59 bp, synthetic construct
  source 1..59: mol_type = other DNA
ttgaagctctaatttgtgagtttagtatacatgcatttacaacgaacgcagaattttcg

SEQ ID NO: 59 - DNA, 59 bp, synthetic construct
  source 1..59: mol_type = other DNA
gtttaataactcgaaaattctgcgttcgttgtaaatgcatgtatactaaactcacaaat

SEQ ID NO: 60 - DNA, 50 bp, synthetic construct
  source 1..50: mol_type = other DNA
gacggtcacagcttgtctgtgtttaaaccgtttaagggcaaatgtactct

SEQ ID NO: 61 - DNA, 50 bp, synthetic construct
  source 1..50: mol_type = other DNA
agagtacatttgcccttaaacggtttaaacacagacaagctgtgaccgtc

SEQ ID NO: 62 - DNA, 59 bp, synthetic construct
  source 1..59: mol_type = other DNA
tgcttcaaaatacctggaattatctgcgtgtttaaacgcttttgttccctttagtgagg

SEQ ID NO: 63 - DNA, 48 bp, synthetic construct
  source 1..48: mol_type = other DNA
ctaaagggaacaaaagcgcggccgcggcaatttggtacaaaaatcacg

SEQ ID NO: 64 - DNA, 46 bp, synthetic construct
  source 1..46: mol_type = other DNA
ctatattatatatatagtaatgtcgtttttgcgaaaccctatgctc

SEQ ID NO: 65 - DNA, 46 bp, synthetic construct
  source 1..46: mol_type = other DNA
gagcatagggtttcgcaaaaacgacattactatatatataatatag

SEQ ID NO: 66 - DNA, 41 bp, synthetic construct
  source 1..41: mol_type = other DNA
gctgaatgggcagttcgaatacctgatgcggtattttctcc

SEQ ID NO: 67 - DNA, 41 bp, synthetic construct
  source 1..41: mol_type = other DNA
ggagaaaataccgcatcaggtattcgaactgcccattcagc

SEQ ID NO: 68 - DNA, 53 bp, synthetic construct
  source 1..53: mol_type = other DNA
gtaagaatttttgaaaattcaatataagtctgaagaatgaatgatttgatgat

SEQ ID NO: 69 - DNA, 56 bp, synthetic construct
  source 1..56: mol_type = other DNA
aatcattcattcttcagacttatattgaattttcaaaaattcttactttttttttg

SEQ ID NO: 70 - DNA, 42 bp, synthetic construct
  source 1..42: mol_type = other DNA
aacacaattgttgatgatcattatagttttttctccttgacg

SEQ ID NO: 71 - DNA, 45 bp, synthetic construct; identical to SEQ ID NO: 55
  source 1..45: mol_type = other DNA

SEQ ID NO: 72 - DNA, 51 bp, synthetic construct; identical to SEQ ID NO: 56
  source 1..51: mol_type = other DNA

SEQ ID NO: 73 - DNA, 41 bp, synthetic construct
  source 1..41: mol_type = other DNA
tatataaactccatgttttaaattgaattgaattgaaatcg

SEQ ID NO: 74 - DNA, 41 bp, synthetic construct
  source 1..41: mol_type = other DNA
gctcatcccgaccttccattaacgaacgcagaattttcgag

SEQ ID NO: 75 - DNA, 41 bp, synthetic construct
  source 1..41: mol_type = other DNA
ctcgaaaattctgcgttcgttaatggaaggtcgggatgagc

SEQ ID NO: 76 - DNA, 52 bp, synthetic construct
  source 1..52: mol_type = other DNA
agacggtcacagcttgtctgtgcggccgcgcttctaataaaccgatgaacgc

SEQ ID NO: 77 - DNA, 52 bp, synthetic construct
  source 1..52: mol_type = other DNA
gcgttcatcggtttattagaagcgcggccgcacagacaagctgtgaccgtct

SEQ ID NO: 78 - DNA, 47 bp, synthetic construct
  source 1..47: mol_type = other DNA
ttttgtaccaaattgccgcggccgcgcttttgttccctttagtgagg

SEQ ID NO: 79 - DNA, 59 bp, synthetic construct
  source 1..59: mol_type = other DNA
aaaggtctcagatcttttccactgcactttgcatgttttagagctagaaatagcaagtt

SEQ ID NO: 80 - DNA, 42 bp, synthetic construct
  source 1..42: mol_type = other DNA
aaaggtctcaaaactctagactttttcgatgatgtagtttct

SEQ ID NO: 81 - DNA, 25 bp, synthetic construct
  source 1..25: mol_type = other DNA
atagaagacgaacattgtacgatac

SEQ ID NO: 82 - DNA, 50 bp, synthetic construct
  source 1..50: mol_type = other DNA
acccaaaaccgataacgccttccgataagtcggtattgttgttgaagatg

SEQ ID NO: 83 - DNA, 43 bp, synthetic construct
  source 1..43: mol_type = other DNA
tcaacaacaataccgacttatcggaaggcgttatcggttttgg

SEQ ID NO: 84 - DNA, 20 bp, synthetic construct
  source 1..20: mol_type = other DNA
aatttctcgtggaagtgacg

SEQ ID NO: 85 - DNA, 24 bp, synthetic construct
  source 1..24: mol_type = other DNA
caatggtctaggtagtggcattcg

SEQ ID NO: 86 - DNA, 47 bp, synthetic construct
  source 1..47: mol_type = other DNA
cgactcactatagggcgaattgggtacgacgggagtggaaagaacgg

SEQ ID NO: 87 - DNA, 46 bp, synthetic construct
  source 1..46: mol_type = other DNA
tcccgttctttccactcccgtcgtacccaattcgccctatagtgag

SEQ ID NO: 88 - DNA, 45 bp, synthetic construct
  source 1..45: mol_type = other DNA
gccaagcacagggcaagatgctttcacagcttgtctgtaagcgga

SEQ ID NO: 89 - DNA, 45 bp, synthetic construct
  source 1..45: mol_type = other DNA
gcatccgcttacagacaagctgtgaaagcatcttgccctgtgctt

SEQ ID NO: 90 - DNA, 25 bp, synthetic construct
  source 1..25: mol_type = other DNA
gattccatgctaccttccatggttg

SEQ ID NO: 91 - DNA, 50 bp, synthetic construct
  source 1..50: mol_type = other DNA
aggaggaaggagggggtgccattatagttttttctccttgacgttaaagt

SEQ ID NO: 92 - DNA, 38 bp, synthetic construct
  source 1..38: mol_type = other DNA
gtcaaggagaaaaaactataatggcaccccctccttcc

SEQ ID NO: 93 - DNA, 50 bp, synthetic construct
  source 1..50: mol_type = other DNA
cgatttcaattcaattcaatttaaaacaaacattgtatatgctcctcaag

SEQ ID NO: 94 - DNA, 51 bp, synthetic construct
  source 1..51: mol_type = other DNA
catatacaatgtttgttttaaattgaattgaattgaaatcgatagatcaat

SEQ ID NO: 95 - DNA, 42 bp, synthetic construct
  source 1..42: mol_type = other DNA
ggaggaaggagggggtgccattatagttttttctccttgacg

SEQ ID NO: 96 - DNA, 38 bp, synthetic construct; identical to SEQ ID NO: 92
  source 1..38: mol_type = other DNA

SEQ ID NO: 97 - DNA, 47 bp, synthetic construct
  source 1..47: mol_type = other DNA
cgatttcaattcaattcaatttaaaacaaacattgtatatgctcctc

SEQ ID NO: 98 - DNA, 41 bp, synthetic construct
  source 1..41: mol_type = other DNA
catatacaatgtttgttttaaattgaattgaattgaaatcg

SEQ ID NO: 99 - DNA, 1659 bp, synthetic construct
  source 1..1659: mol_type = other DNA
atggacttttttgattgttccagatcttccattattccattgaaggcttcctcccaaattgttccagctgattctactaacaagtggggtactgtcgaatctaaccacaactctgctccaactaccccattaaacgacagaatttacgttgaacacgctcacatggtcaaggatttcaagagaatcatgaacgtcgctggtgaagacccatctgaaggtttggctatcatcgatgctgtccaaagattggttgtcgaccatcatttccaagaagaaattcactccatcctacaaaagcataaggaattggctacctctaccaccacacacggtgactgtatgaccacctctttgagattcagattgttgagacaagaaggttactacgtctctgctgatgttttcgaaggtctaaaagatgaagaaggtaagttcgaccaaaacttgagtggtgacatcaagggtttgatggccttgtacgaagcttctcaattctccatggaaggtgaaaacatcttggatgaagccagagactactctgcccgtttattgaatgcttgtgttacccaattgggtcacgatcaagctcgtattgtcgaacacactctgactcacccacaccacaagtctctagccagattcatggccaagaacttcttgagagatttccattgcactaacggttggattgacgacttgaagaagttggccaaagctgacatcgacatggctcaatccactttccaaaacgaagttgttcaaatttctcaatggtggaaggaattaggcttagctgaagaattgaaatttgctcgtgaccaaccagtcaaatggtacatctggaccatgacttgtgacgaagatccatctttctccgaattgagaatcaacttgaccaagccaatctctttcgtctacttgattgatgacatcttcgatgtttatggtaccttgcaagaagtcactgatttcaccgaagctgttcacagatgggaccacgacgccattgaacaattgccataccacatgaagatttgtttcaaggctttggacgatatcaccaacgaaatctcctacaaggtctacaagcaatacggatggaaccctttagactccctcagaaagtcttggggtagattgtgtaacgctttcctaactgaagccaagtggttcgcttctggtcatttggctaaggctgaagaatatttagaaaacggtatcatttcctctggtgttcctgttgttttgttgcacttcttttttcttagtggtgaaggtgttactcaaaagtccgttgaaaccattgacaacactccagacattgtctccgctgcagccgctatcttgcgtttatgggatgatttgggttcagctaaggacgaagaccaagatggtaaggacggttcttacttggcctgttacactaatgaaaacccaggttgttctttggaagatgctgagaagcacgttaagtccaagatctgtgatgaatggaaattgttgaacaaggagtgtttgtctcaaaagaacccattctctggttccttccacagagcttgcttgaatgttgctagaatggttccattgatgtacgaatacgacaagaacagaagattgccaagattggaagaattcttgaagagtatcttgatcaaatga

SEQ ID NO: 100 - DNA, 1803 bp, synthetic construct
  source 1..1803: mol_type = other DNA
atgaacttgccaatgactctaagctccaagtccttattcacttcttccagagcctctatcagctcttctttcaagactatttcccaaattgaaattgctaaaactatcgccaactgtgtcccattgattccagaacaccacaagtggtctattcacgatgtttaccacaaattaagattttccaacactacaaccccaccatttaagcaattgaatcatttgaccaagccatgcaccccaaacgaccacatttctaaggaacacgaaagaaaggtcaaggctttcaagaggattttcaacattgttggtgaagacccaatcgaatccttggtcatcattgacgctgtccaacgtctcggtattgaccatcacttccaagaagaaattaacaccattcttcaagaattgtactacactgaagctaacaacgctcacatcggtggtggtggtggttacttctcccacttgcacgaagtttcgctaagattcagattgttgcgtcaacaaggttgttacgtttctccagaagtctttgactgtttcaaggacaacaacggtaagttcaaagaaaacttgggtggtgacatcaacggtttgatggccttatacgaagcctcccatttgtgtttggaaggtgaaagtctattgcaagaagctcgtgaatgttctgcccaattattaaagaccatcgtcactaacttgaatcactctcaagctaccatggtcgaacacactttgtctcatccacaccacaagtctttctctaaattcaccggtaagaagtacttgtctcacggtttccaagataccaacaatggctggttgaacatcttgaagggtttggctaagattgatttcgacatggctcaatccacttaccaaaaggaaattgtccaaatctctaaatggtgggaagaattgggtttggccaaggaaatgtccttcgccagagatcaaccattaaagtggtacatctggtctatggcttgtatcaccgacccatccttatctgaagaaagaattgacttgactaagtccatctcattcatatacttgattgatgatatcttcgatttgtacggtactcaagacgaattaaccttgtttacccaagttgttaacagatgggactacgatgctagtgaacaattgcctcattacatgaagatttgtttcaaggctttggacgatattatcaacgaaatttcttttaagatctacaagaagcacggatggaacccagttgaatctttgagaaagtcttggggcagactatgctctgcattcttggttgaaggtagatggttcgcttcaggttatgtcccagcttccgaagaatacttgaagaacggtatcatctcttctggtgttcatgttgtctgtgttcaattgttcttcttgttgggtagacaagatataattactaagcaatctgtcgaaatcattgacaacgatccagccatcgtctcctctactgctcaaatcttgagattgtgggatgacctgggttctgctaaggatgaggaccaagatggtcacgacggttcctatttagactactatttgaaagagcaccaaggttgttccgttaaggatgctgaagaacacgttatgtctaagatctctgacgcttggaagcaattgaacaaggaatgtatgacgccaaccccattctctcaatgtttcatcaaggctactttgaacttggctagaatggttcctttgatgtactcttacgacaacaaccaaagattaccatctttggaagataacgttaaatctatcttgtccattgctttgtga

SEQ ID NO: 101 - DNA, 1659 bp, synthetic construct
  source 1..1659: mol_type = other DNA
atggctttcttcggttcctctagatcttcaattattccactaaagactattagtcaaattgttactgctgactccaccaacaagagaggtaccgttgattctaaccacaagtccgctccaaccactcctttgaacgaccgtatctgcaccgaacacgctcacaaggtcaaggatttcaagcaaatcatcaacattgctggtgaagatccatctgaaggcttggctatcattgatgctgttcaaagattgggtgttgaccatcacttccaagatgaaattcacactatcttgcaaaagcattacaccctcgctaccggtacgaccacccatggtgactgtatgatcacttctttgagattcagattacttagacaggaaggttactacgtttctgccgatgttttcgaaggtttaaaggatgaagaaggtaagttcgaccaaaacttgtctggtgacatcaagggtttaatggctttgtacgaagcctcccaattgtccatggaaggtgaaaacatcttggacgaagctagagactactcttccagattgttgaacgaatgtgttacccaattggaccacgaccaagctagaatcgtcgaacacactttgacccacccacaccacaaatctctagcccgtttcatggctaagaacttcttaagagacttccacggtactaacggttggattgacgacttgaagaagttggccaaggttgactttgacatggcccaatctacttaccaaaaggaagtcgtccaaatcagtcaatggtggaaggaattgggtttggctgaagaattgaaattcgctagagatcaaccagtcaagtggtacatctggaccacaacttgtcaccaagacccatctttctcggaattgcgtattaacttaaccaagccaatttctttcgtctacttgattgatgatatctttgatgtctacggtaccccacaagaagttactgacttcactgaagctgtcgatagatgggatcatgatgccatcgaccaattgccatactacatgaagatctgtttcaaggctttagatgacataaccaacgaaatctcttacaaggtttacaagcaacacggttggaacccattggattcattgagaaaatcttggggtagattatgtaacgctttcttgactgaagctcaatggttcgcttctggtcacctgccaaaggccgaagaatacttggaaaatggtatcatcagctccggtgtcccagttgttttgctgcatttgttctttttgttgggtgaaggtgtcactcaaaaatccgttgaaatgattgacaacactccagctattgtctctgctgccgctgctattttgagattatgggacgatttgggctctgctaaggacgaagaccaagatggaaaggatggttcttatttggcatgttacactaatgaaaacccaggttgttccttggaagacgctgaaaagcacgttaagtctaagatttgtgatgaatggaaacaattaaataaagaatgtttgtcccaaaagaacccattctctccatcctttttgaaggcttgcttgaacgtttccagaatggttcctttgatgtacgaatatgacgaaaacagacgtttgccaagattggaagaattcttgaaatccatcttaatcaagtaa

SEQ ID NO: 102 - DNA, 1722 bp, synthetic construct
  source 1..1722: mol_type = other DNA
atggccactgccgctggtccaattgccaccaacaactccccacaaaactctaacgcttacagaaccccaatcgctccatctgttccaatcacccacaagtggtctattgctgaagacttgacttgtatctccaacccatccaagcataacaaccctcaaaccggttacagatctttttctgatgaattatacgttaagtacgaagaaaagttggaagatgtcagaaaggctttgagagaagttgaagaaaacccattggaaggtttagttatgattgacgctttgcaaagattgggaattgattatcacttcagaggtgaaatcggtgctttcttgcagaagcaacaaatcatttcttctactccagatggttacccagaacacggtttatatgaagtctccactttattcagattcttgagacaagaaggtcacaacgttactgctgatgttttcaacaacttcaaggacaaggaaggtcgtttccgttcagaattgtctaccgacatcagaggtttgatgtctttgtacgaagcttctcaattaagaattgaaggtgaagacatcttggaccaagctgctgacttctcctcccaattgttgggtagatggaccaaggatccaaaccatcacgaagccagattggtttctaacactttgactcacccataccacaagtctttggccactttcatgggtcaaaaattgtcctatatgaactgtaagggtccaaactgggacggcgttgacaatttgcaagaactcgctaagatggatttgaccattgttcaatctattcaccaaaaggaagtcttccaagttagtcaatggtggaaagacactggtttggctaatgaattgaagctagccagaaaccaaccattgaagtggtacatgtggccaatggctgccttgaccgacccaagattttctgaagaaagagttgaattgactaagccaatctcttttatctacattattgatgatatcttcgacgtctacggtactattgaagagttgactttgttcaccgatgccgtcaacagatgggaattgtctgctgttgaacaattgccagactacatgaaggtttgtttcaaagctttgtacgacgtcactaatgaaattgcttacaagatatacaagaagcacggtcaaaacccgattgactccttgcaaaagacctgggcttcattgtgtaacgcatttctggtcgaagctaaatggttcgcttccggtcatttgccaaatgctgaagaatacttgaagaacggtatcatctcgtctggtgtccacgttgttttggctcacatgttcttcttattaggtgacggtatcactcaagaatccgtcgatttggtcgacgactacccaggtatctccacctccatcgctaccatcttgagattatccgacgatctaggttctgccaaggacgaagaccaagatggttacgatggttcctacatcgaatgttacatgaaagaacataagggttcttctgttgactccgctagggaagaagttatcagaatgatctctgaagcttggaagtgtttgaacaaggaatgcttgtctccaaacccattctctgaatctttccgtattggttcgttaaacatggctagaatgattccaatgatgtactcttacgatgacaaccacaaccttcctatcttggaagaacacatgaaggctatgatatacaacacctctctataa

SEQ ID NO: 103 - DNA, 1560 bp, synthetic construct
  source 1..1560: mol_type = other DNA
atgaacgtcgaaactaagcacactagaaccatgggtgacatttttgtccaacactctcaaaagttggaactgttgaagacagtcttgagaaatgttgctgaattggacgctcttgaaggtttgaacatgattgatgctgtccaaagattaggtattgactacaacttccaaagagaaattgacgaaatcttacacaagcaaatgtccatagtttctgccagagatgacttgcacgaagtcgctttgagattcagattgttgagacaacacggttacttcgttccagaagatgttttcaacaacttcaaggactccaagggtactttcaagcaagttttgggtgaagacatcaagggcttgatgtctttatacgaagcttctcaattgggaactgaaggtgaagacattttggtggaagctgaaaagttctctggtcacttgttaaagacttctttgtctcacttggatcatcacagagtcagaattgttgctaacactttgcggaacccacatcacaagtctttggctccattcatggctcgtaactttttcgtcacctcccaagctaccaactcttggctaaacttgttgaaggaagttgccaagactgatttcaacatggttagatctctccaccaaaatgaaattgtccaaatgtccaagtggtggaaagaattgggtttagcaaaggaattaaaatttgctagagatcaaccattaaagtggtacatctggtctatggcctgtttgactgacccaaagttgtccgaagaaagagttgaattgaccaagccaatcagtttcgtctacttgattgacgatatcttcgatgtctacggtaccttggatgacttgatcttgttcaccgaagctgttaacagatgggaaatcactgctatcgaccatctgccagactatatgaagatctgtttcaaggctttgtacgacatgactaacgaattctcctccaaggtttacttgaagcatggttggaacccattgcaatctttgaagatttcctgggctagcttgtgcaatgctttcttggttgaggccaaatggttcgcttctggtaagctcccaaagtctgaagaatatcttaagaacggtatcgtctcttccggtgtcaacgttgttttagttcacatgttctttttactaggtcaaaacatcaccagaaagtccgttgaattgttgaacgaaaccccagctattatttcttcttcagctgctattttgcgtttgtgggatgatttgggttctgctaaggatgaaaaccaagatggtaatgacggttcctacgttagatgttacttggaagaacacgaaggttgttctattgaagaagccagagaaaagaccatcaacatgatctctgacgaatggaagaagttgaaccgtgaattattgtctccaaaccctttcccagcctccttcactttggcttcattgaacttggctagaatgatccctttaatgtactcttacgatggtaaccaatgtttgccatccctaaaagaatacatgaaattgatgttgtacgaaaccgtctccatgtaa

SEQ ID NO: 104 - DNA, 1641 bp, synthetic construct
  source 1..1641: mol_type = other DNA
atggccaccaccactacaactatctcaaccacacacaaatggtctatctctgttgctgaagacttgaagtgtttgactcctcattgtactttcaccaacgaaatcttagctaagcaagaagaacaattggaagaagtcagatctgtcttgagaaaggttagagaagaagaagactctctaaagcgtttggttatgatcgacgctttgcaacgtctgggtattgactaccacttcagagaagacatcgaagctgttttgcactcccaatacatgaagtcctcttcccactctttcacttaccaacacgaagatttgtacgaagtttccactagattcagattgttgcgtcaacaaggccacaacgttccaactgatgttttcgataagttcaaggacaaggatggtagatttaagaccgaattgtctgaagacatcagaggtttgatgggtttatacgaagcctcccagttatctattgaaggtgaagatattttggaccaagctgccgacttctctgctcaacaattgaacggttggttgaccagattgggtaaccatcaccaagccaaggttatctctaacactcttggtcatccacaacataaatcattggctaaattcatggctaagaattttttgtctgactacaacggtccaaacgccaatgttttgcaagaactagcgaagatggacttcaacatgtctccatccatgtaccaaaaggaaatgttgcaagtctctaagtggtggaaatccactggtttgggtaacgaattaaagtacgctagaaaccaaccattgaaatggtacttgtggtccatggctactttaacccacccatctttgtctgaacaaagagttgaattgaccaagccaatctctttggtctacattattgacgacatcttcgacgtttatggtaccttggaacaattaattttgttcactgaagctgttaacagatgggaattggccgctgtcaatgaattgccaggttacatgaagatctgtttcaaggtcttgcaagatagtactaatgaaattgcttacggtgtccacaagaagtacggttggaacccaattgatagtttgagaagaacctgggctatcttgtgtaacgctttcttggaagaagctaagtggttcgcttctggtcaattgccaaaggctgaagaatacttaaagaacggtatcgtctccagcggtgtcccagctgtcctcgtccacatgtttttcttgttgggtcacggtatgaacaaggaatctgtcgattttaccatcgataacccagacattatcacttctaccgccaccattttgagattatgggacgatctgggttctgcaaaggatgaaaaccaagacggtcacgatggttcttacgttgattgctatatgaaagaaaacgaaggttccaccgctgaaactgctagaaagcaagttgttgacatgatctctgatgcttggaagagattgaaccgtgaatgtttgtctccaaacagattctccgctaacttcactcaaggttgtctcaacactgccagaatggttccattgatgtactgttacgatgacaaccacaacttgcctattttggaggagcacatgaagtccatgttccacgactccgtcagcttatga

SEQ ID NO: 105 - DNA, 1482 bp, synthetic construct
  source 1..1482: mol_type = other DNA
atgaagaaggaattatccacacgtcactctgaagccttggaagaagtcagaaacctattgaacaatggtccatttaagaacttgcacatggttgacactttgcaaaagttgtgtatcgaccaccacttccaagaagaaattgacatgattttcaagatgtccaacgttcatgactaccaaaccctatacgccttatccttatatttcagaatctttagacaacaaggttactacgttccagctgacgttttcgctaactttaagcaaaaggatggtagattcaaaggtgaaattgctcaagatttgaagggtttattagctttatacgaagcttctcaattatctattccaggtgaagacattttggaggaagctgctgatttctcaagatacttgttggaacaaaagatcccatttttgggtcaagaagaagccctcaaggttaacaacaccttggaacactcctaccaaaagatcccatctaacttcagattgaagatcttcatcaagcactactctggtaccaccatgtctgacttggctatgctggaattggctaaggccaagtctgttcacgctactgaagttgaacaattctccagatggtggaaggatctaggtttggctcaagaattgaaattggccagaaaccaaccattgcactggtacttgtggccaatggctggtttgactgacttgtctttgtctgaaatcagaattgacttgaccaagccaatcgctttggtcttcattattgatgacatcttcgatgtctacggtactttggaccaattgattttattcactgaagctgttaccagatgggattccaataacttggaacaattgccatacaatttgagaacttgtgttcaagctgtctttgatgttactcacgaaatctctgataaaatttacaacaagtacggtttcaaccctattgaattcttgaagcaaacttggactgatttgtgtgaagctttcttagtcgaagcaaagtggttcaccaaaggttacatgccaaaggctgaagattatttaaagaacggtgccgtctccaccggtgctcacgttgtgattgtccacatgttcttcttgttgggtggtgccacctccaaggaaactgctcaaatcattgacgaacacaagggtatcacttcttgcttagccaagatcttgcgattgtgggacgatttgggttctgctaaggacgtcaaccaagacggtcatgacggctcatacgtcacttactatatgaatgaaaactctggatgttccatccaaaacgctcgtgaacatgttatgaagatgatcatcaacacctggaaacaattgaacaaagaatgtttgtctccaaacccattctctgccactttcaccaaggcttgtttgaacttggctagaatgattcctttgatgtacaactacgatgaaaaccatagtttgccattgatcaaggactacattaactccatgttctaa

SEQ ID NO: 106 - DNA, 52 bp, synthetic construct
  source 1..52: mol_type = other DNA
gatatcgacaaaggaaaaggggcctgttcatttgatcaagatactcttcaag

SEQ ID NO: 107 - DNA, 46 bp, synthetic construct
  source 1..46: mol_type = other DNA
gaatttttgaaaattcaatataaatggacttttttgattgttccag

SEQ ID NO: 108 - DNA, 46 bp, synthetic construct
  source 1..46: mol_type = other DNA
gacaaaggaaaaggggcctgttcacaaagcaatggacaagatagat

SEQ ID NO: 109 - DNA, 48 bp, synthetic construct
  source 1..48: mol_type = other DNA
aagaatttttgaaaattcaatataaatgaacttgccaatgactctaag

SEQ ID NO: 110 - DNA, 52 bp, synthetic construct
  source 1..52: mol_type = other DNA
atcgacaaaggaaaaggggcctgtttacttgattaagatggatttcaagaat

SEQ ID NO: 111 - DNA, 44 bp, synthetic construct
  source 1..44: mol_type = other DNA
atttttgaaaattcaatataaatggctttcttcggttcctctag

SEQ ID NO: 112 - DNA, 47 bp, synthetic construct
  source 1..47: mol_type = other DNA
caaaggaaaaggggcctgtttatagagaggtgttgtatatcatagcc

SEQ ID NO: 113 - DNA, 42 bp, synthetic construct
  source 1..42: mol_type = other DNA
gaatttttgaaaattcaatataaatggccactgccgctggtc

SEQ ID NO: 114 - DNA, 49 bp, synthetic construct
  source 1..49: mol_type = other DNA
atcgacaaaggaaaaggggcctgtttacatggagacggtttcgtacaac

SEQ ID NO: 115 - DNA, 52 bp, synthetic construct
  source 1..52: mol_type = other DNA
taagaatttttgaaaattcaatataaatgaacgtcgaaactaagcacactag

SEQ ID NO: 116 - DNA, 46 bp, synthetic construct
  source 1..46: mol_type = other DNA
gacaaaggaaaaggggcctgttcataagctgacggagtcgtggaac

SEQ ID NO: 117 - DNA, 50 bp, synthetic construct
  source 1..50: mol_type = other DNA
aaagtaagaatttttgaaaattcaatataaatggccaccaccactacaac

SEQ ID NO: 118 - DNA, 48 bp, synthetic construct
  source 1..48: mol_type = other DNA
cgacaaaggaaaaggggcctgtttagaacatggagttaatgtagtcct

SEQ ID NO: 119 - DNA, 52 bp, synthetic construct
  source 1..52: mol_type = other DNA
gtaagaatttttgaaaattcaatataaatgaagaaggaattatccacacgtc